European Patent Specification EP 3 253 400 B1, published January 18, 2023. Title: Oleanoyl peptide composition and a method of treating skin aging. Applicant: Majeed, Muhammed Nagabhushanam Kalyanam Chandramouli Renukeshwar H Sood, Rattan Prakash, Subbalakshmi Tathapudi,Susmitha Anand. The sequence listing filed with the application follows.

SEQUENCE LISTING (1 sequence)

SEQ ID NO: 1 - protein, 5 aa, Artificial Sequence
  Description of Artificial Sequence : Synthetic peptide
KTTKS